European Patent Specification EP 3 973 984 B1, published January 7, 2026. Title: Glycoconjugate Vaccine. Applicant: London School of Hygiene and Tropical Medicine. The sequence listing filed with the application follows.

SEQUENCE LISTING (17 sequences)

SEQ ID NO: 1 - protein, 697 aa, Pseudomonas aeruginosa
MKKIWLALAGLVLAFSASDQNATGGDQNATGGDQNATGGDQNATAAEEAFDLWNECAKACVLDLKDGVRSSRMSVDPAIADTNGQGVLHYSMVLEGGNDALKLAIDNALSITSDGLTIRLEGGVEPNKPVRYSYTRQARGSWSLNWLVPIGHEKPSNIKVFIHELNAGNQLSHMSPIYTIEMGDELLAKLARDATFFVRAHESNEMQPTLAISHAGVSVVMAQAQPRREKRWSEWASGKVLCLLDPLDGVYNYLAQQRCNLDDTWEGKIYRVLAGNPAKHDLDIKDNNNSTPTVISHRLHFPEGGSLAALTAHQACHLPLEAFTRHRQPRGWEQLEQCGYPVQRLVALYLAARLSWNQVDQVIRNALASPGSGGDLGEAIREQPEQARLALTLAAAESERFVRQGTGNDEAGAASADVVSLTCPVAKDQNRTKGECAGPADSGDALLERNYPTGAEFLGDGGDVSFSTRGTQNWTVERLLQAHRQLEERGYVFVGYHGTFLEAAQSIVFGGVRARSQDLDAIWRGFYIAGDPALAYGYAQDQEPDARGRIRNGALLRVYVPRWSLPGFYRTGLTLAAPEAAGEVERLIGHPLPLRLDAITGPEEEGGRVTILGWPLAERTVVIPSAIPTDPRNVGGDLDPSSIPDKEQAISALPDYASQPGKPPREDLKDQNATGGDQNATGGDQNATGGDQNATVD

SEQ ID NO: 2 - protein, 225 aa, Francisella tularensis
MKKIWLALAGLVLAFSASGTDQNATGGDQNATGGDQNATGGDQNATGTMKKIIELSLLSLSIAGLASCSTLGLGGSDDAKASAKDTAAAQTATTEQAAAVSKPTAKVSLNKLGQDKIKATVYTTYNNNPQGSVRLQWQAPEGSKCHDTSFPITKYAEKNDKTWATVTVKQGNNFCSGKWTANVVYDKEVIASDSINIDQNATGGDQNATGGDQNATGGDQNATVD

SEQ ID NO: 3 - protein, 590 aa, Francisella tularensis
MKKIWLALAGLVLAFSASGTDQNATGGDQNATGGDQNATGGDQNATGTMVSREDFIMTINKLSLTDELLNNFGGSTEVDSVLKNIDFDVSDDASKVLSLSTDYNARNLMALSLVLANNDNINNYNQKYIQKVITVIDKLIDLQVNSIISNDEFRALEQEWLKVQEVCQEDYDNVEVSILDVKKEELQYDFERNLYDISSSDFFKKVYVSEFDQYGGEPYGAILGLYNFENTTNDIIWLTGMGMVAKNSHAPFIASIDKSFFGVKDLSEITHIKSFEALLEHPRYKEWNDFRNLDVAAYIGLTVGDFMLRQPYNPENNPVQYKLMEGFNEFVDYDKNESYLWGPASIHLVKNMMRSYDKTRWFQYIRGVESGGYVKNLVACVYDNKGILETKSPLNVLFADYMELSLANIGLIPFVSEKGTSNACFFSVNSAKKVEEFVDGFDSANSRLIANLSYTMCISRISHYIKCVIRDKIGSIVDVESIQKILSDWISEFVTTVYQPTPLEMARYPFRNVSIEVETIPGKPGWYSCKINVIPHIQFEGMNTTMTIDTRLEPELFGTNNNDQNATGGDQNATGGDQNATGGDQNATVD

SEQ ID NO: 4 - protein, 171 aa, Francisella tularensis
MKKIWLALAGLVLAFSASGTDQNATGGDQNATGGDQNATGGDQNATGTMNIRPLQDRVLVRRAEEEKKSAGGIILTGSAQEKPSQGEVVAVGNGKKLDNGTTLPMDVKVGDKVLFGKYSGSEVKVGDETLLMMREEDIMGIIADQNATGGDQNATGGDQNATGGDQNATVD

SEQ ID NO: 5 - protein, 718 aa, Francisella tularensis
MKKIWLALAGLVLAFSASGTDQNATGGDQNATGGDQNATGGDQNATGTMGKIIGIDLGTTNSCLAIMDGKTAKVIENAEGHRTTPSVVAYTDSGEILVGQAAKRQAVTNPDNTFFAIKRLIGRKYDDKAVQEDIKKKVPYAVIKADNGDAWVATKEGKKMAPPQVSAEVLRKMKKTAEDYLGEPVTEAVITVPAYFNDSQRQATKDAGKIAGLEVKRIINEPTAAALAYGVDSKKGEQTVAVYDLGGGTFDISIIEIADVDGDNQIEVLSTNGDTFLGGEDFDLALMNYLIDEFKKEQGIDLHNDKLALQRVREAAEKAKVELSSAQQTDVNLPYITADATGPKHLNIKVTRAKFESLVSDLVMRSLEPCKKALEDAGLSKSDITEVLLVGGQTRMPLVQEKVKEFFGKEPRKDVNPDEAVAVGAAIQGGVLAGDVKDILLLDVTPLSLGIETMGGVMTKLIERNTTIPTKKSQVFSTAEDNQPAVTIHVLQGEREMASANKSLGRFDLADIPPAPRGMPQIEVTFDIDANGILNVSAKDKATGKEQNIVIKSSSGLSEEDIEKMVQDAEANAEADKKFHDLVTARNTADNLIHSSRKAIQELGDKVTAAEKEKIEEACKELEAATKGDDKQAIESKTKALEEAFAPIAQKAYAEQAQAAVAQGGAKAEEPKKEEDVVDADFEDVEDDKKDQNATGGDQNATGGDQNATGGDQNATVD

SEQ ID NO: 6 - protein, 620 aa, Francisella tularensis
MKKIWLALAGLVLAFSASGTDQNATGGDQNATGGDQNATGGDQNATGTMAAKQVLFSDEARAKMLDGVNTLANAVKVTLGPKGRNVVLDKSFGTPTITKDGVSVAKEIELEDKFENMGAQIVKEVASKTADVAGDGTTTATVLAQALLTEGLKAVAAGMNPMDLKRGIDKATARLVEELKALSKPCSDPKSIEQVGTISANSDATVGKLIADAMAKVGKEGVITVEEGKGFEDELDVVEGMQFDRGYLSPYFATNQENMTTDLENPYILIVDKKISNIRDLLPILEGVSKSGRALLIIAEDVESEALATLVVNNMRGVVKVCAVKAPGFGDRRKAMLEDIATLTGATFVSEDLSMKLEETNMEHLGTASRVQVTKDNTTIIDGAGEKEAIAKRINVIKANIAEANSDYDREKLQERLAKLSGGVAVIKVGAVTEAEMKEKKDRVDDALHATRAAVEEGIVAGGGVALIRAQKALDGLTGENDDQNYGIALLRKAIEAPLRQIVSNAGGESSVVVNQVKANQGNYGYNAANDTYGDMVEMGILDPTKVTRSALQHAASIAGLMITTEAMIGEIKEAAPAMPMGGGMGGMPGMMDQNATGGDQNATGGDQNATGGDQNATVD

SEQ ID NO: 7 - DNA, 18852 bp, Francisella tularensis
atgaattatcatataaaagaagtattctggtcaattattttatcattcttaaaatcacaaaaaggtatacataccaatgatgaagccaaattaagattgtttattgaagctgtattttatgtgttacgtacaggctgtcaatggagaatgttaccattttattatggtaaatatagatcaatacataagcgttttaaagattggtgtgataaagatatattttctagattatttaaatcagtacaaaaccctgatttacaagaagtcatgcttgattcaacaatagcaagagcacatgcttgtgctacgggatatgataaagatgataaccaagcaattggtagatcagttggtaggataaccactaaaatccatgctatgactgatgctttaggtaatccaatagaaatattgttgtcagaggataaaactcatgatagtaaagtagctatagatttactaaaaaatgtatataatacaaaagttatcgctgatagagcatatcattctaatgaaatcaggcagcatattcaaggtatatcctctgaagctgttatcccttgtaaatcaaatactctaaaccatataccttttgatagtcatgtatataaagaaagacatttgatagagaatttcttttctaaaattaagcattttagaagagtattctctagatttgataaaaccattttagcatatataggaatgattaaattagcttgtacttttatttggttacgatgaatatttatttttgtgcacagaacctaatttgcatttttgtgcacaaagaaaatttttttgatataatagactttaataggatattttctaaaaattaacaaatgtctttctacgataatagaacgcttaatttcgtggtaataatagttttaactattattactgttaattggactttctatattttcaagcaagatgttaatttacattttttacttgcattagttttgctgagatgcttgtcatcttttttactacttagagattatatggctagttggcgtaagtcgactcaaaaaacttttttacgtaaggcttttattaatttgccagtatttttcatagtggcattatttttttatggcaaagtcactttttcgttgatattctctgagtttttattttatgtttttttgatcagtttaagtgtctacttttattggtatttgatgaacagaggatcagtggataaaagtaaaactgcggttatttatggtgcaggtgctgcaggaacaaagattgctcaagaacttgcttctgctggttatcgcatcaaatgttttgttgatgacaatgaaactttacaaaaaagaagtattgatagtaaaaaggttctatctaaagctgaattaacaaaactattgctatctagtagatttgaccttttggttattgcattgccaagaaatgcaaaccaagtagtcaaaaatatatataaagaatttgaaaaggattttaatcagattagaattatgccgcctcttgaggaaattcttcaagatgagaattttatgtcacagttgaagcctgtttcactctatgatctattagcgcgtgatactaagagtttagataaagaatctatctctaattttatcaaaaataaggtggtgctagtcacaggagctggaggtagtataggttctgaaatagtacatcaatgtatcaagtatcaggcaaaagagttgatattggttgatcatagtgagtttaacttatataaaattactgaggagtgtagtcattttaatatcaatagtgtgctatgttctgtttgtgatagaaaagcattggctgaggtttttcaaaagtatactccaaatatagtatttcatgctgctgcctacaagcatgttcccttagttgaggagaatatctctagagcaattagaaataatatcttaggtactaagaatgctatagatctggctatagaagctggtgttgagtcatttatattgatttccactgataaagcagtgcgaccaacgaatgttatgggggctaccaagagagtttgtgagctgtatttacagaatgttgatcccaaaaataccaagcttgctgcagtgcgttttggtaatgtgcttggtagtagtggcagtgtgattccaaaatttgaagagcaaataagaaaaggtggtcctgttacagttactcatcctgaaattacacgttattttatgttgataccagaagcttgtgaactggtcctacaagctggtgctattgcaaaaaattcagaggtctttgtcttagatatggggcaacctgtcaagattattgatcttgctaaacaatttattagactttctggtagaggtgatattgatattaaaatagttggtttgcgtccaggagagaaactttacgaagagcttttgatagaggaagatgatgttagtaccgactataaagatatttttattggtagaaggactttttacgatattaatactctaaaccaagatattgaatcgttgatcaaggatgatgttgatcagcttgtgatattaaagaaaattgttccggaatttgaacatagattgaatgggtagtggttttatgttttatgaggtttttaaaagattgcttgatattttactttcttttatggggttgttgttattaagtcctattttcttaattattatttttatgataaagaaagattcaaaaggacctatattttttaaacaaaagcgctatggtaaagataagcaatttttttacatatataagtttagaactatgtatgttgatactccaaaagatatgccaacgcacatgttacaggatccatcgaaatgtataactaaggttggaggatttttaaggaaatcatctttagatgagttgccacaaattataaatattctaaaaggtgaaatgagcatcgtgggtccaagaccagcattatggaatcaagatgacttaatagcacaaagagataagtatggggcaaatgctgtgcctgtgggactgactggctgggcacagattaatggtagggatgaattaccaatacctgataaagctaaacttgatggtgattatgtaaaaaataaaagtacatggtttgatttaaaatgtatttttttgacagtattttctgtttttgccaaaaagggcgtcgttgagggtggtactggagctttaggtaacaaagaggatttaaagtagtatgaaaaaaagaatcttagttacaggtttgagtagctatattggtaactcatttgcggctaaatataactcagattttagtatcgataaaatatctttgcgcgatgtttcgtgggcaaatatagacttaagtggttatgatgctgtattgcatgtcgctggaattgcccatacttcaaaggatcctaaactaaaagaaaaatactataaaataaatacgcaattaacttatgatctggcaaaacaagctaaagatcaaggtgttcgacagtttgtgtttttaagtagtattatagtttatggtgatagtgcgccaataggtcaacaaaaagttataactaaatataccgaacctaaaccagatgatttttatggagatagtaagcttcaaactgaaattaagctaaatagcctggctagtgatgactttaatattgctataatcagaccaccaatggtatatggagaaggctcaaaaggcaactatccaaagttggttaaacttgcaaagtatacttttatttttcctaatattaataaccaaagaagtgttatatctatagataatttatctaaagagattgcagaaataattttgcaaactaaacatggagtttttctacttcaagataatgaatatttttgcacttcacagtttataaaaaactatagaaaagatgttttaggtaagagaacttatctgacaaaaatttttaatccaattataagattgcttgctaaaaaagtagattttattaataaagtttttgggaatttgacttatgagaagtaagttattattcatagctaatgattttgatattgtaatatatcgtttcagaagagaagtaatcgagtcttttgctgctaaagagtatgagatagtactagtaacaccatattctaagaaagcagaggttttttgtaaaagtcttggtgttaagtatataaatgttgatatagatagacgaggcaaaaatccttttaaggatttgcttcttttatttaactatttcaaaataataaaaaaagaaaaacctgattacatttttagctatacaattaaaccaaatttgtatgttgggttagtgaatttgttttttaggaagaagttttatccaaatgtaacaggcttaggaagtgtttttgctaatcatggtattgttcagaagtttataatatctttatataagttatcatttaaaagcaccacaaaagtattctttcagaatgagcaaaataaaaagttatttatagctaagaaaataatcagtggagaaaaatcaatattattaccaggttctggggtaaacttagatgaaaataaatatgttgactatcctaaagaccaaggaatattaaaattcgtttttcttggccgaataatgaaagaaaaggggatttatgaattgttagaagcctttgctatacttgagaaaaaatataaaaatattagtcttgacatttatggtttttgtgatgaaaataaatctaattttatgggaaaggttaatacgataaaatcagtaaaattttatggttttactgataatactaaagaaaaaatagctagtgcacatgcagttgttttgccatcttaccatgaaggaatgtcaaatgtgctgttagaagcagctgcgataggtagacctgtaattgcgtcagatattcctgggtgtagagaaatttttgatgatggtctctctggcttatcatgtaaccctaatgatgtgagttctttacgtaactcattagagcagtttataaatatgtcgtatactgataaaatagctatgagctataaagctagagctaagatagaaaaagattttgatagaagtattgttgtcaatgcatacttacagcaaaattaataataagggtttaaattatgagtttatatgaggatatagtcgctaaaagagaaaaggtttcattggttggcttgggttatgttggtttaccaatagctattgcatttgcaaaaaaaatagatgtgttaggatttgatatttgtgaaacaaaagttcaacattataaggatggttttgatccaacaaaagaagtaggagatgaggctgtcagaaatacgacaatgaaatttagttgtgatgaaacaagtcttaaagagtgtaaatttcatattgttgcagttcctacaccagttaaagcagataaaactcctgatttgacgccgattattaaggcaagtgagacggttggtaggaatcttgtcaaaggcgcttatgttgtgtttgaatcaactgtttatcctggtgttacagaagatgtttgcgtaccaatacttgaaaaagagtctggcttgaggtctggtgaagatttcaaagttggttactctcctgagaggataaatcctggtgataaggttcataggttagaaacaattatcaaagtagtatctggtatggatgaagagtctttagatactatagcaaaagtttatgagctagtagtagacgcaggagtttatagagctagtagtataaaagtggctgaagctgctaaggttatagaaaactctcaaagagatgttaatatagcttttgttaatgagttatcgataatatttaatcagatgggtattgatactctagaggttttagcagcagctgcaactaaatggaatttcttaaactttaagcctggtcttgttggtggacattgtattggtgttgacccatattacctaacgtacaaggcagctgagcttggatatcattctcaggtaatattatctggtcgtaggataaatgatagtatgggtaaatttgtagttgagaatttagtcaaaaaactgatatctgcagatatacctgttaagcgagctagagtagcaattttcggctttacttttaaagaagactgtcctgacactaggaatactcgagttatagatatggtaaaagagctcaacgagtatggtatagagccatatattatagatccggtagctgataaagaagaggctaaacatgagtatggacttgagtttgatgatctaagtaaaatggtcaatctagatgcgatcattattgctgttagtcacgaacagtttaaagatataacaaagcaacagtttgataggctatatgcgcataattctagaaagattatatttgacatcaaaggtagtttagataaatctgagtttgaaaaagattatatttattggagattgtagtggcttacgataatgttaaatttcctcatggttcgttttttttggtgactggaggtgcgggttttattggctctaatttatgtgaagttttacttagtaagggttatagagttaggtgtttagatgatctctcaaatggtcactatcacaatgttgagccgtttttaactaattctaattatgagtttataaaaggtgatattagagatttagatacttgcatgaaagcttgtgaaggtattgattatgttctacatcaagctgcttggggaagcgtaccaagaagtattgagatgccattagtgtatgaagatataaatgttaaaggtgcattaaatatgcttgaagcggctagacaaaataacgttaaaaaatttgtctatgcttctagttcatcagtatatggtgatgagccaaatttacctaaaaaagaaggtagagaaggaaatgttttatcaccctatgcatttacaaagaaagctaatgaagagtgggcgagactatacacaaagttatatggtctagatacttatggtctaagatattttaatgttttcggtagaagacaagatcctaatggtgcgtatgcagcagttatacctaaatttatcaaacagttattaaatgatgaagcgccaactataaatggagatggtaaacagtcgagagattttacatatatagagaatgttattgaggcaaatcttaaagcatgtttagcagatagtaagtatgccggagagtcttttaatatagcttatggaggtagagagtatcttatagatttgtactataatctttgtgatgccttgggtaaaaaaatagagccaaattttggtccagatagagcgggtgatattaagcatagtaatgctgatatttcgaaggctaggaatatgctcggatataatccggaatatgattttgaattaggcataaagcatgctgttgagtggtatttaattaattaaatggtattttaatcaagtgtacataaaaaaagtgtcttttaaaattttatatttatatttactagctttttgtattatttttagtttagaatttaaatttgctatattgaatattatagtttatcttccggcttgtattttgggttttttagctcttaaaaaactatttgtcggaaatattgttaagaaacaattagctttcctttttttctttttctttttatcaatgatttatttaataatagtccaaataatcttacttgatgcagcatcattgtttcctcagtttttatttaacattttgatcgcgataggtttttgtaactttatttttgtttcatatgataataatgaaaattatttttttaatatgtctaaaataatattttttgttactttcttacaatctatttttgtatttctttcaaggtattatatatttttaaatgattggatattcttttttttagtgaaaaaagggaatattgagatttcgaatgttattgaatataagttaagagtattcggacttagtaacgctggaggggatggtttaggattttcaattactataggattatgtttttctatattttattttatcaaatatattaaaggtaaatctatatttaccaaacttatgctgtttgtacctttaattcttattgtgttttctaatattttcatatctagaacatcactcttaacttcttcacttatattgttaataacaatattttatatatatattaaaaaagaaaaattactgtttattataatattggcgctattctttttatcaatatggatattgttcaaattaaatttgaatttgagttgggcttttgaaaatatttactcgtacattcaatctggcgatttttcacatggaagtctaagtgttttaatcaataaaatgctttttgtgccagataaccttttgacttggatatttggttgtgaggatgttagtaatactgatattggttatattaaatatttatactattatgggattatatttagtatgtttttttatattcttattattttcttgtactttgaaatgagaaaatgttttatattttcagagtatcgatcattatttctattgttgttaatagtatgtttagtttttcaagcaaaaataatttttttgacagtaggattatttactaaattaaccattatattatttattttttctcttaaagaaaacagctttacaactaggagtgtgatttgaaaaggtttgtacatttaataataaaccttaaccaaggtggtgctgaaacaatgctttataaactttgcaaatctatggataagtcaatatatcatattacgattatatcacttatgggtaggggagtatttgcaaataagttagaagcttatggtgttaaagtttatacattaaatttaaataaatttaatgtactatttgtattgtttaaatatattaagattatcagaagaataaagcctgatgttattcatgcttggatgtatcatgcaaatgtaatttctatattatgcaagcctttttatagaaagactaaatatataaatagtataagaatgggattggagaattatgatggtcataagaatcttacaaagtttatgataaagttgaatgcaaaattttctaagttctcagatttaacattaaataattcaaagaaatcattagaagatcatcaaaatataggttttaaaaaccaatgctttatagcaaatggttttgataaagatgtttttaaaccgagctttttaaagtatgaaaaatttcgtttaaataatgatttagatgataatgttaaaattataggtatcatagcaagaaatcatgctgataaaaatatttctcgtttcttacaaatagctaatttattgttaaaaagtaatcctagtttacggtttttaattgctggaagagagtgttcgaaaatagatataggtagttatctagataacaaaagtaatgtaaataagttttttgtatttgaatctgtggattctagtgaatacttaccagtattagatttatatttgtctacatcaaaagttgaaggttttccaaatatacttgcagaagccatgctatgtgaagttcctattgttgcttctaatgttggagattgtaaagatatacttaatggatacggtgaagtttttgagcttagtcaaggtaataaagaaataatagaaaagattatgaaagttttagaaacaacggtagtcatgaaaaagcgcatgagagaatatataataaataattttagtatagaagctattttggaaaaacacgaaaaactttatcatgagggcagtgtctaatgtgtggagtagtaggcttttactcatttaataaagaagaaggttttgactcaataattaatcaatcattgctttctataaagcatagagggtcggatgatagtgggtattggtgcgacaatcaagttactctggggcatactagattatcaatacacgatataactaatgcgggacatcagccaatgttatctaatagcggtaatactgctattgtgtttaatggagaaatatataattacttatccataaaaaatcagctattaagtgaatattcaaatcttaaatttaaaagtaacagtgatactgaggttttggtcaatgctattgaactttggggtatagataaaactttagaaaaatgcataggaatgtttgcttttggagtttacagtagaaaaactagttgcttaatactagctagagatagatttggcgagaagccattatattttggtatccaaaatggtattttgggttttgcatcagaattgaaggcacttaagccattaaaggaatgtggctggaggtttgatatagatagagatgctttagcaacatatatgaggtatgcttatgtaccaacaccatactctatttataaaaatatatctaaactaaatgtaggtagttacataaaatttgatgctaaaggtaatagtaaagagtataaatattgggattctaaaaaagtactagattcagaaaaatataaagattcgtatgatcaagcaatcctagatttagaaattaagcttaaaagtacactatcaatacaaatgcagtcagatgttcctctaggagcatttttatccggaggaattgactcaacaactgtagttgctcttatgcaaagtatgtctaaagataagataaacacttttagtataggttttaatcaaaaagaatataatgaagctgagcatgcaagagcagtagcaaaacatataggtacaaaccacacagatatgtatgttacagaaagagatgctcttgatgtaataccaaaacttgctggaatatatgacgagccctttgctgattcatcacaaataccaacgtatcttgtgagtaaaatagctaagtcgaaagtaacagttgcactatcaggtgacgctggtgatgagctctttggcggttataatagatactttttagcaccaaatattgctaaaaaaatcaaatttgctaagttacttaaatatgcaccagatgcttggataaaaaaagctgagatattaaattttggtaagttcgctttattagcagataaactactaaaactaaaaagagttctcgaaaaagcaaaaacaaataaagagctttatgtactactttgttcacaaataaatgatactagctttgtgttaggagcaaaagagtatgatatattaagagataagaatatttatgatattccacaattatctttccaagagtggatgatgtttgttgattctaatacatatatgatagatgatatattggttaaggttgatagagcagctatggctaactctctagagacaagagtgccatttttagatcataatatttatgaatttgcttattccttaccaattgactataaaatacaacgaggtaacggaaaaagaattttgaaagatttgttatataaatatgtgccagaaagtttggtcaataggtctaagatggggtttggtattccgcttgctaaatggttaagagaagatttacgagagtgggcagataatttactggattatagtaaaatagacaagcaaggttacttaagtcctgaggtggtgcaaaaatattggcaagagcatttgagtggtaaaagaaattggcaagcaatattatggaatattctaatttttcaggagtggttagataatgagtaaagtaaatgtaacaaaaccatacttaccagatataaataaatataaaagctatgtaaataaaatatacaaaaatggatggcttactaataatggtccgttagtgcaagagctagaaaaaagacttgcaaagtatctaggtgttaaaaatatagttttagtatcaaatggtacaattgcattagaaatcgcgtatagagcgttaggagtcaaaggaagtgcaattactactccattttcatttgttgctactacatcttcattggtttctaacaatgtaaaaccagtgtttgttgatattgatgagaatactctaagtatagacgtctctaaaattaagtatgctattgaagaggatacttcagctattgtgccagttcatgtgtttggaaatggttgtgaagttgaaaaaatagacatgctggctaaaaaacataacttaaaagttatttatgatgcagcacatgcttttgatgttaagtataagggtgagagtatattaaactatggtgatatttcgacattaagttttcatgcaacaaagatttttcattctattgaaggaggtgcgcttatcattaatgatgatagtcttgttgaaaaagttcgttatttcattaattttggtatagaaagctcagaatcaataccttacttaggtactaatgctaaaatgaatgaatttgaggcggctatgggactttgtgttctagatgatattatagaaattaagagcaaaaggaaagttattacagagatatatgaggctgggttagatggattggtaaagtttcaagaacagaatcagcattctagtaggaattatagctattttccagtaatatttaggactgaggaggaacttctcagagtacagaaagcactaatacaaaatgatataatatcgcgtagatatttttatccatcattagatagtcttagttatatagagccaaagcagtatatgccaatctcaagagatatatctaaaagaatattatgtttgccaatttatgcagagttagaagacgataaaattaataaaataattaataatatcaaagaggtttcctcatgaaaaaaatatttgttgttacagataatagaactattctaagtgattttaaaaatatcattggtagtaaaaatgatgtagaggttgattatttttgtagtttcaagagtcaaacttcttttgccaaagaaatatataacagtgagattaagccaatagatatgaaaaaaaatggcaatgatcttattggtaagtatgatttaggtttttcttgtcattcgaaacaattatttccagcaaaattagttaattcagtattatgtataaatattcatcctggacttaatccatataatagagggtggtttccacaggtcttctctattataaataaactacctataggagcaactattcatgtgatggatgaagagatagatcatggagatataatcattcaggaagaagttgaagttaattctttcgaaaactcttttgatgtttatgctaaagttcaaaaaaaagaagttgagttgttcactaaagtcatagatgatattttgaataataagttcactcgaatcaaacctaactccgaaggcaactataattcaattcatgattataaaaacatgtgtgaaattgatttagataaaatagtaacaatgcgggaagcaattgactatctaagggctatgacacaccctccatataaaaatagttatttcattgatgagcatggaaataaagtatttgttgctcttgaacttgaaaagataagttagaaaaatgagccttaaaaaaaatacaatatcaaattatataacacaactatatactagcttaattggtattgttatacttcctttgtatttacaacatttaagtcatgatgcatttggtctgattggtttttttacagtttttcaaacgtggttacggttgttggatgttggtataacaccaactttatcaagagaagtggctcatgttagaggtagtactgatgactatcattacttacgcaagttggttagatcgttagagctatttttcattattgttggtgttctggtatttattgtaattagtacacattcaaggtatatatccacctcttggttacatataggctcgctagatgctgatagtgtaagtgtatgtattgcacttatgggtttaatgtttgcattaagatgggtgtctgatctatatggtggtggtttgcgtggctttgaaagacaggttctttataataatttaagtatcatacaaacgacactacagtttattggtggattattatttatctgctatgtgtctactaatattatgtattattttgtatatcagacaataattgcgatactatatctagtatgtattgcaattgcattttataaaatactaccatcatcatttagcgtgggtttaaggtttgattttaaaataattagaaaagtgcttccatttgcactaggcattgcatattctacaacagtttggattattgtcactcaatctgataaattagtgttctcacatgtattaccattatctgagtatggttatttatctttattgatagtgatatctagtgctgttacgatattgtcctctccgattagcatagctattcagcctagaatgacaatgctattagcccaacaaaatgtaaaaggaatggaaagcttatatttaaaatcatccttgatctcaattacttttttatctgctgtagtaacatgtgttttgatgtattctcatcagctgttgcagtcatggacaggaagtatggaaattgctaattggggtagtaatatcttaaatatatatgttttatcagcatctattatttgtataatatcatttcaatattttttacagtatgcttatggtaagttaaagctacataatacatataatacaattagtttagtattttttgctcctatagttatatatactgcttataattatggagtgtatactacagcactattatggcttggatatgctatagtggggctgataatctggatgcctattgtacaccatgtatttgctaaaggtatcaataggtatttttttataaatttagcagttattactatagtatgttttttattatcgttaatatttaagggttggtatatttatccaagtaaaattgggttggtagaattaatattgattgggtttgcatttttatttatacaaatttgtatagagtatgttttgtttcggtacaaggttttgaggtgtatagatgattaaagtttcagtatgtgtgatgacatacaatcaagaaaagtatattggtcaatgtttagagtctttggttactcaagagactgattttgactttgagataatcgttggagatgatttttctacagatggtacaagagatgttattcaagagtatcaaaaaaagtatccggatatcataaagccagtttttagagataagaatgtgggaattactgaaaatattaaagaaatctattttgttgcaaatggtgagtatatagctcatatggatggtgatgattatgcattgcctggtaaacttcaaattcaggctgattttttggataataatccaagatgtacgggagtttttcataatataaatatactctatccaaatggtaatatacaacatagtaggtttgcttgttcaaataagagtatattcaatttatcagacactttacgcggagttgctgttggtgcaaatagttcaaaaatgttcagaacatcggttttggatgatttgattttaccggatatagagcttctagattattattttcatgttataacagcagaaaaaggttatttaagttttttaaattctaatgaatcctatagtgtgtacagaaaaggtattggtatcacatctaagtctaaggaaaaaatctataatacttatgctggattatttgaatattttttggatagatatcctgaagagaaattaaatatttgtatccctgttgtgcaaatgataatttcggctattaaagggagatgttttattagtgctattcgtctattcaaaattttaattagatcaagatgtattccattagtaagttggtttaaatatagatttgaaaaataaatatcatttagaggattatgtgaaatgaagggaataattctagctggtggcagtggtacaaggctatatccacttaccttgggtgttagcaaacagctgctacctgtttatgacaagccattgttatactatccactatctgtgcttatgcttgcaggtattagggagatattaattatctctacagtgcgtgatatctcacttatccaagagcttcttggtgatggttcacaatttggtatacagttgagttataaaatccagccatcaccagatgggcttgctcaagcatttattcttggtgaggagtttttggcgggtgactcagcttgtttgatattaggagataatatctactatggtcaaggtatgactacaatgctagagtctgcaagagcacagtgtggaggtccagctggtggcgcttgtgtttttggttattatgttaatgatccgcatagatatggtatagtcgaatttgataagcaaaaaaatgtaatttcggtagaggaaaagccacagaatcctaagtcacactatgctatcacaggtttatatttttatgataataatgttgttgagtatgctaaacaagtcaaaccatctgcacgtggtgagctagagattacttcacttaatgagttatatctaaaagaaaataagctaaatgtcgaactcttagggcgtggctttgcttggcttgatgctggtacgcatgattcattgctagaggcaggtcaatatgtcgcaactattgagaaaagacaagggcttaaaattgcatgtttggaagaaattgcatggcgtaaaggctttatctcaacacaacaagttctagctcaagctgaaaaactttctaagacagagtatggtcagtatctgaagaatttaattaaggatggtttataaattaatccgtcatacccatgaaggtgggtatctcataaaagttggatatgttttggagattccaatctgcgcagtaatgacaggtttggtaatatatagcgatgttttacaatgactaaaaatggttttatgtatattcttacaaataaggataatactgttctgtacatagttgtaacatctaatttgataaaaagaatgtatgagcataaacatagccttgcagatggttttactaaaaatataatgttaataagttagtttattttgaaatttatgaagatataaaagcagcaattctgtgagaaaagcagttgaaaaaatgaaacagatcttggaaagaacgaattattaatgagatgaatccgaattggaatgatttatatgaattaatatgtgagtaaaacttttgtcttactggtgcagataggtatctctaaatatcagatgtgattgggagattaccgcctacgcggtaatgacaagtttatgcggtaatgatagtttagtgagagaatgactagtcactataggaatgatgatgtaatgaggaatgaaaaaatgaactacaaaccaaaaaatatcctagtaacaggtgcggcgggatttattggtagtaactatgtgcgtatgatgttatcacgctatagtgatatcaaaataatctcgtatgataagcttacttatgcgggtagtttagataatctaaaagacttgaataatgaacataaccatacttttataaaaggtgatatttgtgatgaagttttagtatatcaaacactgaaagaatataaaattgatacgatagtacattttgctgcagaatcgcatgttgataattcaattgctaatccaaaggtatttttagaaacgaatgtgataggtacatttacacttttagattgtgctaaaaggtattggttagatgagctaggtttagaagaaactagttgtaggtttcatcatgtatctactgatgaggtatatggtaccttggcaaaagatgaaccagcctttactgagattaaggcttatgagccaaattcaccgtattcggcatctaaggcgggatctgatcatatttctagagcatatcatcatacctataaacttccggtaacaatttcaaattgttcaaacaactatggaccataccaacatcgagagaaattaatccctgtagtgataaatagttgtataaactacaagcctattcctgtttacggagatggttcgaatattcgagattggctatatgtagaagatcactgcgatgctatccagacaattgttgagaaaggagtggttggagaggtttataatattggtggtattaatgaagttgataatctaaccttggtaaaaactatctgtaaactaatggatgaatataaaccagaaaatgctccacattctaacttaatcacatttgtggaagatagaaaaggacatgattggcgttatgctattgataacagcaagattcagaatgagttaggatggaagccatcacaagattttgataagatgtttagacaaactattgagttttatctatagcttaaatatttatcttatgagtatctctaaaaaatcaatttaatttatttttgtgttaaaaagtagtgttcgcaagaatatagttaatccgaaagatatttgtagaaaaagatatttgtagaaatgttataatgtctaataaaaatgccatcatatagccaagattttagagacatcgtaattaataaacatgaagaaggtatgacggagttcgagctgagtaagttttttaacatagataagcgtacagttgtttcatggatagagttttataaaagaaccggagattatagttcaaagcaaggagttggttgtggcagagtcgctagctttaccgataaaacattgattgaacagtatttgatagatcatccagatgcaagtgcattagatataaaagaagcattagcccctgatattccaagaagtacattttatgattgtcttaatagacttggttttagttttaaaaaaagactccaaaatataagcaaagaaaagaacatgaaaggttggagtatatagaaaaactaaaagaaatagccaataaatttgatgtacaaatattatatctacctccgtactctccagatttaaatcctattgaaaaggtttgggctaactattaa

SEQ ID NO: 8 - DNA, 2142 bp, Campylobacter jejuni
atgttgaaaaaagagtatttaaaaaacccttatttagttttgtttgcgatgattatattagcttatgtttttagtgtattttgcaggttttattgggtttggtgggcaagtgagtttaatgagtattttttcaataatcagttaatgatcatttcaaatgatggctatgcttttgctgagggcgcaagagatatgatagcaggttttcatcagcctaatgatttgagttattatggatcttctttatccgcgcttacttattggctttataaaatcacacctttttcttttgaaagtatcattttatatatgagtacttttttatcttctttggtggtgattcctactattttgctagctaacgaatacaaacgtcctttaatgggctttgtagctgctcttttagcaagtatagcaaacagttattataatcgcactatgagtgggtattatgatacggatatgctggtaattgttttgcctatgtttattttattttttatggtaagaatgattttaaaaaaagactttttttcattgattgccttgccgttatttataggaatttatctttggtggtatccttcaagttatactttaaatgtagctttaattggactttttttaatttatacacttatttttcatagaaaagaaaagattttttatatagctgtgattttgtcttctcttactctttcaaatatagcatggttttatcaaagtgccattatagtaatactttttgctttattcgccttagagcaaaaacgcttaaattttatgattataggaattttaggtagtgcaactttgatatttttgattttaagtggtggggttgatcctatactttatcagcttaaattttatatttttagaagtgatgaaagtgcgaatttaacgcagggctttatgtattttaatgtcaatcaaaccatacaagaagttgaaaatgtagatcttagcgaatttatgcgaagaattagtggtagtgaaattgtttttttgttttctttgtttggttttgtatggcttttgagaaaacataaaagtatgattatggctttacctatattggtgcttgggtttttagccttaaaaggggggcttagatttaccatttattctgtacctgtaatggccttaggatttggttttttattgagcgagtttaaggctataatggttaaaaaatatagccaattaacttcaaatgtttgtattgtttttgcaactattttgactttagctccagtatttatccatatttacaactataaagcgccaacagttttttctcaaaatgaagcatcattattaaatcaattaaaaaatatagccaatagagaagattatgtggtaacttggtgggattatggttatcctgtgcgttattatagcgatgtgaaaactttagtagatggtggaaagcatttaggtaaggataattttttcccttcttttgctttaagcaaagatgaacaagctgcagctaatatggcaagacttagtgtagaatatacagaaaaaagcttttatgctccgcaaaatgatattttaaaaacagacattttgcaagccatgatgaaagattataatcaaagcaatgtggatttgtttctagcttcattatcaaaacctgattttaaaatcgatacgccaaaaactcgtgatatttatctttatatgcccgctagaatgtctttgattttttctacggtggctagtttttcttttattaatttagatacaggagttttggataaaccttttacctttagcacagcttatccacttgatgttaaaaatggagaaatttatcttagcaacggagtggttttaagcgatgattttagaagttttaaaataggtgataatgtggtttctgtaaatagtatcgtagagattaattctattaaacaaggtgaatacaaaatcactccaattgatgataaggctcagttttatattttttatttaaaggatagtgctattccttacgcacaatttattttaatggataaaaccatgtttaatagtgcttatgtgcaaatgttttttttaggaaattatgataagaatttatttgacttggtgattaattctagagatgctaaggtttttaaacttaaaatttaa

SEQ ID NO: 9 - protein, 713 aa, Campylobacter jejuni
MLKKEYLKNPYLVLFAMIILAYVFSVFCRFYWVWWASEFNEYFFNNQLMIISNDGYAFAEGARDMIAGFHQPNDLSYYGSSLSALTYWLYKITPFSFESIILYMSTFLSSLVVIPTILLANEYKRPLMGFVAALLASIANSYYNRTMSGYYDTDMLVIVLPMFILFFMVRMILKKDFFSLIALPLFIGIYLWWYPSSYTLNVALIGLFLIYTLIFHRKEKIFYIAVILSSLTLSNIAWFYQSAIIVILFALFALEQKRLNFMIIGILGSATLIFLILSGGVDPILYQLKFYIFRSDESANLTQGFMYFNVNQTIQEVENVDLSEFMRRISGSEIVFLFSLFGFVWLLRKHKSMIMALPILVLGFLALKGGLRFTIYSVPVMALGFGFLLSEFKAIMVKKYSQLTSNVCIVFATILTLAPVFIHIYNYKAPTVFSQNEASLLNQLKNIANREDYVVTWWDYGYPVRYYSDVKTLVDGGKHLGKDNFFPSFALSKDEQAAANMARLSVEYTEKSFYAPQNDILKTDILQAMMKDYNQSNVDLFLASLSKPDFKIDTPKTRDIYLYMPARMSLIFSTVASFSFINLDTGVLDKPFTFSTAYPLDVKNGEIYLSNGVVLSDDFRSFKIGDNVVSVNSIVEINSIKQGEYKITPIDDKAQFYIFYLKDSAIPYAQFILMDKTMFNSAYVQMFFLGNYDKNLFDLVINSRDAKVFKLKI

SEQ ID NO: 10 - DNA, 28 bp, Artificial Sequence
  Primer FTfragment2rev
ggatcattaatagctaaatgtagtgctg

SEQ ID NO: 11 - DNA, 32 bp, Artificial Sequence
  Primer Oant1ftfwd
ttttgaattctacaggctgtcaatggagaatg

SEQ ID NO: 12 - protein, 5 aa, Artificial Sequence
  Glycosylation site
  MISC_FEATURE (1)..(5): Glycosylation site wherein X is any amino acid except proline
DXNXS

SEQ ID NO: 13 - protein, 5 aa, Artificial Sequence
  Glycosylation site
  MISC_FEATURE (1)..(5): Glycosylation site wherein X is any aminoacid except proline
DXNXT

SEQ ID NO: 14 - protein, 5 aa, Artificial Sequence
  Glycosylation site
  MISC_FEATURE (1)..(5): Glycosylation site wherein X is any amino acid except proline
EXNXS

SEQ ID NO: 15 - protein, 5 aa, Artificial Sequence
  Glycosylation site
  MISC_FEATURE (1)..(5): Glycosylation site wherein X is any aminoacid except proline
EXNXT

SEQ ID NO: 16 - DNA, 2133 bp, Campylobacter sputorum
atgtcaaattttaatttcgctaaatttctaaataaattacctagactttctaaacatactattttaatgattgttttagctgtttgttttgggatattttgcagattttactgggtagtttgggctagtgcttatccgcattttatatggaatgatcagcttatgataagcacaaatgacggatatgcatttgctgagggcacaagagatatgatagctggttttcatcaaccaaacgatctttcttactatggctcatctctttcgacgcttagcatgtggttatataacattttgccattttcattagaaactatacttttgtatatgagtacatttttatctccactcttagctgtgcctttgatacttataggtaaagaactaaacgcttcaaaagcgggttttatagctgcacttctagctattattgcaaatagttattataatagaacaatgagtggatattacgatacggatatgctaaatatcactcttcctatgatggttttttggagcataacaagacttgttcaaagaaaagagagagtaaatttaatatttattccggtttttatggcgatatatggatggtggtatccatcttcttactcactattacttgccatgattggaatgttttttttatataccattgtttttgaaagatacgaaaaactaaactatgaagctatggtttttatgattttagcaatcacaagcttttctatacaaattaaatttattatagttattgttttgtatgctttaatctatttttaccaaagattttttgataaaaaagtaatatttgcattaattatggcttcgttaatatgctttatatggcttggcgggctaaaccctatactttttaacattaaattttatatatttagagacattgcagatagcggtgatgctgtttttaaatttttcaatgtaaatcaaacaataagagaaagttctgcgatagattttaacacagttgtaactaggattagcgggcatttaatagtatttttggtatctattataggatatattttatttataaaaaacaataaaattttactactaactttaccgattctgtttttgggtcttatgtcatttaaaagtggtttaagatttacaatatactcagttccagtaatggctcttggttttggctattttgttatgtattgttttgcaaaaatagatataaaagatcgttttttaggttatgtgtttttatttgttgtaacatttagtgcattatatccatctttaaaacatatttatgattataaagtatttcctgtttttacacatagcgaagttgaaagtttggataatttaaaaaatattgcaaaaagagaagattatgtgctttcttggtgggattatggttatccgatcagatattattcagatgtaaaaactctcatagatggaggaaaacatcttggaagtgataacttcgccgttagctttgcacttggaagcgatcaaaatagctctgcaaatatggcaagattagaagttgaatatacagaaaaaaattatgaagaaaaatttggattaaatttaaaaaagatgatgaaagattataatgctacaaatgttaatgagtttttattatcattaaaagatgaaaatttaactctgccaaagcaaacaagagatatttattactatttaccagatagaatgatatacatatatccgatagtgctagatttttctagacttgatttgacaacagggcaagaatttgcccagccgttttttatggttagtgagagattttcagctacaaatgataatcaaataatgttaaataacaatgtcatattaagtaatgatggcactaaattatcgataaatggcaactcttatagtgtaaatacatatgttgaaacaagttatgatcaaaacgaaaaattaaatgtaaattattttaacatagatccaaatagcaatttttatgtgatttttatgaaagattatttgagaattttggttttagataaaactttgtatgatagtgcgtatattcaactttttgtattagaaaattatgataaaaatttatttgaaccagtgattttaaacggatcaactaaaatttataaactcaaaaaatga

SEQ ID NO: 17 - protein, 710 aa, Campylobacter sputorum
MSNFNFAKFLNKLPRLSKHTILMIVLAVCFGIFCRFYWVVWASAYPHFIWNDQLMISTNDGYAFAEGTRDMIAGFHQPNDLSYYGSSLSTLSMWLYNILPFSLETILLYMSTFLSPLLAVPLILIGKELNASKAGFIAALLAIIANSYYNRTMSGYYDTDMLNITLPMMVFWSITRLVQRKERVNLIFIPVFMAIYGWWYPSSYSLLLAMIGMFFLYTIVFERYEKLNYEAMVFMILAITSFSIQIKFIIVIVLYALIYFYQRFFDKKVIFALIMASLICFIWLGGLNPILFNIKFYIFRDIADSGDAVFKFFNVNQTIRESSAIDFNTVVTRISGHLIVFLVSIIGYILFIKNNKILLLTLPILFLGLMSFKSGLRFTIYSVPVMALGFGYFVMYCFAKIDIKDRFLGYVFLFVVTFSALYPSLKHIYDYKVFPVFTHSEVESLDNLKNIAKREDYVLSWWDYGYPIRYYSDVKTLIDGGKHLGSDNFAVSFALGSDQNSSANMARLEVEYTEKNYEEKFGLNLKKMMKDYNATNVNEFLLSLKDENLTLPKQTRDIYYYLPDRMIYIYPIVLDFSRLDLTTGQEFAQPFFMVSERFSATNDNQIMLNNNVILSNDGTKLSINGNSYSVNTYVETSYDQNEKLNVNYFNIDPNSNFYVIFMKDYLRILVLDKTLYDSAYIQLFVLENYDKNLFEPVILNGSTKIYKLKK